European Patent Specification EP 3 665 200 B1, published April 16, 2025. Title: HER3 BINDING AGENTS AND USES THEREOF. Applicant: University of Saskatchewan Mohammad, Ayman Elsayed Fonge, Humphrey Barreto, Kris Geyer, Clarence Ronald. The sequence listing filed with the application follows.

SEQUENCE LISTING (122 sequences)

SEQ ID NO: 1 - protein, 11 aa, Artificial Sequence
  Synthetic construct
RASQGISNYLA

SEQ ID NO: 2 - protein, 7 aa, Artificial Sequence
  Synthetic construct
AASSLQS

SEQ ID NO: 3 - protein, 9 aa, Artificial Sequence
  Synthetic construct
QQYGWLPLT

SEQ ID NO: 4 - protein, 2 aa, Artificial Sequence
  Synthetic construct
SY

SEQ ID NO: 5 - protein, 17 aa, Artificial Sequence
  Synthetic construct
VISYDGSNKYYADSVKG

SEQ ID NO: 6 - protein, 13 aa, Artificial Sequence
  Synthetic construct
TDPYSLGGYYFDY

SEQ ID NO: 7 - protein, 107 aa, Artificial Sequence
  Synthetic construct
DIQMTQSPSSLSASVGDRVTITCRASQGISNYLAWYQQKPGKAPKLLIYAASSLQSGVPSRFSGSRSGTDFTLTISSLQPEDFATYYCQQYGWLPLTFGQGTKVEIK

SEQ ID NO: 8 - protein, 122 aa, Artificial Sequence
  Synthetic construct
EVQLVESGGGLVQPGGSLRLSCAASGFTFSSYGMHWVRQAPGKGLEWVAVISYDGSNKYYADSVKGRFTISRDNSKNTLYLQMNSLRAEDTAVYYCARTDPYSLGGYYFDYWGQGTLVTVSS

SEQ ID NO: 9 - protein, 9 aa, Artificial Sequence
  Synthetic construct
QQYGWLPLK

SEQ ID NO: 10 - protein, 9 aa, Artificial Sequence
  Synthetic construct
QQYGWLPLT

SEQ ID NO: 11 - protein, 9 aa, Artificial Sequence
  Synthetic construct
QQYGWLPPT

SEQ ID NO: 12 - protein, 8 aa, Artificial Sequence
  Synthetic construct
QQYAYPLT

SEQ ID NO: 13 - protein, 8 aa, Artificial Sequence
  Synthetic construct
QQYGYPLT

SEQ ID NO: 14 - protein, 8 aa, Artificial Sequence
  Synthetic construct
QQYSYPLT

SEQ ID NO: 15 - protein, 8 aa, Artificial Sequence
  Synthetic construct
QQYGSPLT

SEQ ID NO: 16 - protein, 8 aa, Artificial Sequence
  Synthetic construct
QQYSFPLT

SEQ ID NO: 17 - protein, 9 aa, Artificial Sequence
  Synthetic construct
QQYTTHPLT

SEQ ID NO: 18 - protein, 9 aa, Artificial Sequence
  Synthetic construct
QQAGYRPLT

SEQ ID NO: 19 - protein, 20 aa, Artificial Sequence
  Synthetic construct
ARAPSYSYGSYHYYYYYFDV

SEQ ID NO: 20 - protein, 21 aa, Artificial Sequence
  Synthetic construct
ARAPSYSYGSYHYYYYYYFDV

SEQ ID NO: 21 - protein, 21 aa, Artificial Sequence
  Synthetic construct
ARAPSYSYGSYHYYYYYYFDY

SEQ ID NO: 22 - protein, 21 aa, Artificial Sequence
  Synthetic construct
ARSPSYSYGSYHYYYYYYFDV

SEQ ID NO: 23 - protein, 21 aa, Artificial Sequence
  Synthetic construct
ARAPSYHFGVHSFYYYYYFDV

SEQ ID NO: 24 - protein, 20 aa, Artificial Sequence
  Synthetic construct
ARSPYAYFGSHHYYYYYFDV

SEQ ID NO: 25 - protein, 21 aa, Artificial Sequence
  Synthetic construct
ARSGSYYHYGWHYYYYYYFDV

SEQ ID NO: 26 - protein, 21 aa, Artificial Sequence
  Synthetic construct
ARSPSYYYGHDYFYYYYYFDV

SEQ ID NO: 27 - protein, 20 aa, Artificial Sequence
  Synthetic construct
ARSSPYFYGYSYYYYYYFDV

SEQ ID NO: 28 - protein, 20 aa, Artificial Sequence
  Synthetic construct
ARAGYYVYGASAYYYYYMDV

SEQ ID NO: 29 - protein, 18 aa, Artificial Sequence
  Synthetic construct
ARGGSAWYVSYYYYYFDV

SEQ ID NO: 30 - protein, 16 aa, Artificial Sequence
  Synthetic construct
ARAGYASPYYYYYFDY

SEQ ID NO: 31 - protein, 17 aa, Artificial Sequence
  Synthetic construct
ARAGYASPYYYYYYFDY

SEQ ID NO: 32 - protein, 16 aa, Artificial Sequence
  Synthetic construct
ARAGYAPGYYYYYFDY

SEQ ID NO: 33 - protein, 17 aa, Artificial Sequence
  Synthetic construct
ARAGYASPYYYYYYFDV

SEQ ID NO: 34 - protein, 17 aa, Artificial Sequence
  Synthetic construct
ARGGYASPYYYYYYFDV

SEQ ID NO: 35 - protein, 17 aa, Artificial Sequence
  Synthetic construct
ARGGYASPYYYYYYFDY

SEQ ID NO: 36 - protein, 17 aa, Artificial Sequence
  Synthetic construct
ARAGYYSPYAYYYYFDY

SEQ ID NO: 37 - protein, 18 aa, Artificial Sequence
  Synthetic construct
ARGGSHSSYPGYYYYFDY

SEQ ID NO: 38 - protein, 19 aa, Artificial Sequence
  Synthetic construct
ARGGSHSSYPGYYYYYFDY

SEQ ID NO: 39 - protein, 16 aa, Artificial Sequence
  Synthetic construct
ARGGYSSYGYYYYFDY

SEQ ID NO: 40 - protein, 17 aa, Artificial Sequence
  Synthetic construct
ARGGYSSYGYYYYYFDY

SEQ ID NO: 41 - protein, 18 aa, Artificial Sequence
  Synthetic construct
ARGGYSSYPGYYYYYFDY

SEQ ID NO: 42 - protein, 19 aa, Artificial Sequence
  Synthetic construct
ARAGHVPGPWGYYYYYFDY

SEQ ID NO: 43 - protein, 18 aa, Artificial Sequence
  Synthetic construct
ARYYGYDPSHYYYYYFDY

SEQ ID NO: 44 - protein, 15 aa, Artificial Sequence
  Synthetic construct
ARTDPYSLVGYYFDY

SEQ ID NO: 45 - protein, 14 aa, Artificial Sequence
  Synthetic construct
ARTDPYSLVYYFDY

SEQ ID NO: 46 - protein, 15 aa, Artificial Sequence
  Synthetic construct
ARTDQYSLGGYYFDY

SEQ ID NO: 47 - protein, 15 aa, Artificial Sequence
  Synthetic construct
ARTDSYSLGGYYFDY

SEQ ID NO: 48 - protein, 15 aa, Artificial Sequence
  Synthetic construct
ARTDPYSLGGYYFGY

SEQ ID NO: 49 - protein, 15 aa, Artificial Sequence
  Synthetic construct
ARTDPYSLGGYYFNY

SEQ ID NO: 50 - protein, 15 aa, Artificial Sequence
  Synthetic construct
ARADPYSLGGYYFDY

SEQ ID NO: 51 - protein, 15 aa, Artificial Sequence
  Synthetic construct
ARTDPYSLGGYYFDY

SEQ ID NO: 52 - protein, 15 aa, Artificial Sequence
  Synthetic construct
ARTDPYSLGGHYFDY

SEQ ID NO: 53 - protein, 15 aa, Artificial Sequence
  Synthetic construct
ARTDPYSLGGYYFDV

SEQ ID NO: 54 - protein, 15 aa, Artificial Sequence
  Synthetic construct
ARTDRHSLGGYYFDY

SEQ ID NO: 55 - protein, 9 aa, Artificial Sequence
  Synthetic construct
ARGGYYFDY

SEQ ID NO: 56 - protein, 11 aa, Artificial Sequence
  Synthetic construct
ARHGSYAAFDY

SEQ ID NO: 57 - protein, 20 aa, Artificial Sequence
  Synthetic construct
ARAPSTLTVLPLLLLLLLRR

SEQ ID NO: 58 - protein, 15 aa, Artificial Sequence
  Synthetic construct
ARTDPYSLGGYYFDY

SEQ ID NO: 59 - protein, 15 aa, Artificial Sequence
  Synthetic construct
ARTDPYSLGGHYFDY

SEQ ID NO: 60 - protein, 15 aa, Artificial Sequence
  Synthetic construct
ARTDPYSLGGYYFDV

SEQ ID NO: 61 - protein, 15 aa, Artificial Sequence
  Synthetic construct
ARTDRHSLGGYYFDY

SEQ ID NO: 62 - DNA, 52 bp, Artificial Sequence
  Synthetic construct
  misc_feature (25)..(28): n is three nucleotides encoding Y, S, G, T, A, P, H, R, E, F, W, V or L
ttcgcaacttattactgtcagcaannnncctctgacgttcggacagggtacc

SEQ ID NO: 63 - DNA, 45 bp, Artificial Sequence
  Synthetic construct
  misc_feature (21)..(21): n is three nucleotides encoding Y, S, G, T, A , P, H, R, E, F, W, V or L
  misc_feature (22)..(22): n is three nucleotides encoding A, G, D or Y
ccgtctattattgtgctcgcnnttcgactactggggtcaaggaac

SEQ ID NO: 64 - DNA, 46 bp, Artificial Sequence
  Synthetic construct
  misc_feature (21)..(22): n is three nucleotides encoding Y, S, G, T, A, P, H, R, E, F, W, V or L
  misc_feature (23)..(23): n is three nucleotides encoding A, G, D or Y
ccgtctattattgtgctcgcnnnttcgactactggggtcaaggaac

SEQ ID NO: 65 - DNA, 47 bp, Artificial Sequence
  Synthetic construct
  misc_feature (21)..(23): n is three nucleotides encoding Y, S, G, T, A, P, H, R, E, F, W, V or L
  misc_feature (24)..(24): n is three nucleotides encoding A, G, D or Y
ccgtctattattgtgctcgcnnnnttcgactactggggtcaaggaac

SEQ ID NO: 66 - DNA, 48 bp, Artificial Sequence
  Synthetic construct
  misc_feature (21)..(24): n is three nucleotides encoding Y, S, G, T, A, P, H, R, E, F, W, V or L
  misc_feature (25)..(25): n is three nucleotides encoding A, G, D or Y
ccgtctattattgtgctcgcnnnnnttcgactactggggtcaaggaac

SEQ ID NO: 67 - DNA, 49 bp, Artificial Sequence
  Synthetic construct
  misc_feature (21)..(25): n is three nucleotides encoding Y, S, G, T, A, P, H, R, E, F, W, V or L
  misc_feature (26)..(26): B is three nucleotides encoding A, G, D or Y
ccgtctattattgtgctcgcnnnnnnttcgactactggggtcaaggaac

SEQ ID NO: 68 - DNA, 50 bp, Artificial Sequence
  Synthetic construct
  misc_feature (21)..(26): n is three nucleotides encoding Y, S, G, T, A, P, H, R, E, F, W, V or L
  misc_feature (27)..(27): n is three nucleotides encoding A, G, D or Y
ccgtctattattgtgctcgcnnnnnnnttcgactactggggtcaaggaac

SEQ ID NO: 69 - DNA, 51 bp, Artificial Sequence
  Synthetic construct
  misc_feature (21)..(27): n is three nucleotides encoding Y, S, G, T, A, P, H, R, E, F, W, V or L
  misc_feature (28)..(28): n is three nucleotides encoding A, G, D or Y
ccgtctattattgtgctcgcnnnnnnnnttcgactactggggtcaaggaac

SEQ ID NO: 70 - DNA, 52 bp, Artificial Sequence
  Synthetic construct
  misc_feature (21)..(28): n is three nucleotides encoding Y, S, G, T, A, P, H, R, E, F, W, V or L
  misc_feature (29)..(29): n is three nucleotides encoding A, G, D or Y
ccgtctattattgtgctcgcnnnnnnnnnttcgactactggggtcaaggaac

SEQ ID NO: 71 - DNA, 53 bp, Artificial Sequence
  Synthetic construct
  misc_feature (21)..(29): n is three nucleotides encoding Y, S, G, T, A, P, H, R, E, F, W, V or L
  misc_feature (30)..(30): n is three nucleotides encoding A, G, D or Y
ccgtctattattgtgctcgcnnnnnnnnnnttcgactactggggtcaaggaac

SEQ ID NO: 72 - DNA, 54 bp, Artificial Sequence
  Synthetic construct
  misc_feature (21)..(30): n is three nucleotides encoding Y, S, G, T, A, P, H, R, E, F, W, V or L
  misc_feature (31)..(31): n is three nucleotides encoding A, G, D or Y
ccgtctattattgtgctcgcnnnnnnnnnnnttcgactactggggtcaaggaac

SEQ ID NO: 73 - DNA, 65 bp, Artificial Sequence
  Synthetic construct
  misc_feature (21)..(27): n is three nucleotides encoding Y, S, G, A, F, W, H, P or V
ccgtctattattgtgctcgcnnnnnnntactactactactttgactactggggtcaaggaaccct

SEQ ID NO: 74 - DNA, 60 bp, Artificial Sequence
  Synthetic construct
  misc_feature (21)..(28): n is three nucleotides encoding Y, S, G, A, F, W, H, P or V
  misc_feature (38)..(38): n is three nucleotides encoding G or Y
  misc_feature (39)..(39): n is three nucleotides encoding M or F
  misc_feature (43)..(43): n is three nucleotides encoding V or Y
ccgtctattattgtgctcgcnnnnnnnntactactacnngacntggggtcaaggaaccct

SEQ ID NO: 75 - DNA, 61 bp, Artificial Sequence
  Synthetic construct
  misc_feature (21)..(29): n is three nucleotides encoding Y, S, G, A, F, W, H, P or V
  misc_feature (39)..(39): n is three nucleotides encoding G or Y
  misc_feature (40)..(40): n is three nucleotides encoding M or F
  misc_feature (44)..(44): n is three nucleotides encoding V or Y
ccgtctattattgtgctcgcnnnnnnnnntactactacnngacntggggtcaaggaaccct

SEQ ID NO: 76 - DNA, 64 bp, Artificial Sequence
  Synthetic construct
  misc_feature (21)..(29): n is three nucleotides encoding Y, S, G, A, F, W, H, P or V
  misc_feature (42)..(42): n is three nucleotides encoding G or Y
  misc_feature (43)..(43): n is three nucleotides encoding M or F
  misc_feature (47)..(47): n is three nucleotides encoding V or Y
ccgtctattattgtgctcgcnnnnnnnnntactactactacnngacntggggtcaaggaaccct

SEQ ID NO: 77 - DNA, 67 bp, Artificial Sequence
  Synthetic construct
  misc_feature (21)..(30): n is three nucleotides encoding Y, S, G, A, F, W, H, P or V
  misc_feature (43)..(43): n is three nucleotides encoding G or Y
  misc_feature (44)..(44): n is three nucleotides encoding M or F
ccgtctattattgtgctcgcnnnnnnnnnntactactactacnngacgtttggggtcaaggaaccct

SEQ ID NO: 78 - DNA, 68 bp, Artificial Sequence
  Synthetic construct
  misc_feature (21)..(31): n is three nucleotides encoding Y, S, G, A, F, W, H, P or V
  misc_feature (44)..(44): n is three nucleotides encoding G or Y
  misc_feature (45)..(45): n is three nucleotides encoding M or F
ccgtctattattgtgctcgcnnnnnnnnnnntactactactacnngacgtttggggtcaaggaaccct

SEQ ID NO: 79 - DNA, 69 bp, Artificial Sequence
  Synthetic construct
  misc_feature (21)..(32): n is three nucleotides encoding Y, S, G, A, F, W, H, P or V
  misc_feature (45)..(45): n is three nucleotides encoding G or Y
  misc_feature (46)..(46): n is three nucleotides encoding M or F
ccgtctattattgtgctcgcnnnnnnnnnnnntactactactacnngacgtttggggtcaaggaaccct

SEQ ID NO: 80 - DNA, 72 bp, Artificial Sequence
  Synthetic construct
  misc_feature (21)..(33): n is three nucleotides encoding Y, S, G, A, F, W, H, P or V
  misc_feature (49)..(49): n is three nucleotides encoding M or F
ccgtctattattgtgctcgcnnnnnnnnnnnnntactactactacggangacgtttggggtcaaggaaccct

SEQ ID NO: 81 - DNA, 73 bp, Artificial Sequence
  Synthetic construct
  misc_feature (21)..(34): n is three nucleotides encoding Y, S, G, A, F, W, H, P or V
  misc_feature (50)..(50): n is three nucleotides encoding M or F
ccgtctattattgtgctcgcnnnnnnnnnnnnnntactactactacggangacgtttggggtcaaggaaccct

SEQ ID NO: 82 - DNA, 76 bp, Artificial Sequence
  Synthetic construct
  misc_feature (21)..(35): n is three nucleotides encoding Y, S, G, A, F, W, H, P or V
ccgtctattattgtgctcgcnnnnnnnnnnnnnnntactactactacggaatggacgtttggggtcaaggaaccct

SEQ ID NO: 83 - protein, 248 aa, Artificial Sequence
  Synthetic construct
SDIQMTQSPSSLSASVGDRVTITCRASQGISNYLAWYQQKPGKAPKLLIYAASSLQSGVPSRFSGSRSGTDFTLTISSLQPEDFATYYCQQYGWLPLTFGQGTKVEIKGGGGSGGGGSGGGGSEISEVQLVESGGGLVQPGGSLRLSCAASGFTFSSYGMHWVRQAPGKGLEWVAVISYDGSNKYYADSVKGRFTISRDNSKNTLYLQMNSLRAEDTAVYYCARTDPYSLGGYYFDYWGQGTLVTVSS

SEQ ID NO: 84 - protein, 238 aa, Artificial Sequence
  Synthetic construct
SDIQMTQSPSSLSASVGDRVTITCRASQGISNYLAWYQQKPGKAPKLLIYAASSLQSGVPSRFSGSRSGTDFTLTISSLQPEDFATYYCQQYGWLPLTFGQGTKVEIKGGGGSEISEVQLVESGGGLVQPGGSLRLSCAASGFTFSSYGMHWVRQAPGKGLEWVAVISYDGSNKYYADSVKGRFTISRDNSKNTLYLQMNSLRAEDTAVYYCARTDPYSLGGYYFDYWGQGTLVTVSS

SEQ ID NO: 85 - protein, 226 aa, Artificial Sequence
  Synthetic construct
SDIQMTQSPSSLSASVGDRVTITCRASQGISNYLAWYQQKPGKAPKLLIYAASSLQSGVPSRFSGSRSGTDFTLTISSLQPEDFATYYCQQYGWLPLTFGQGTKVEIKRTVAAPSVFIFPPSDSQLKSGTASVVCLLNNFYPREAKVQWKVDNALQSGNSQESVTEQDSKDSTYSLSSTLTLSKADYEKHKVYACEVTHQGLSSPVTKSFNRGECGGSDYKDDDDK

SEQ ID NO: 86 - protein, 242 aa, Artificial Sequence
  Synthetic construct
EISEVQLVESGGGLVQPGGSLRLSCAASGFTFSSYGMHWVRQAPGKGLEWVAVISYDGSNKYYADSVKGRFTISRDNSKNTLYLQMNSLRAEDTAVYYCARTDPYSLGGYYFDYWGQGTLVTVSSASTKGPSVFPLAPSSKSTSGGTAALGCLVKDYFPEPVTVSWNSGALTSGVHTFPAVLQSSGLYSLSSVVTVPSSSLGTQTYICNVNHKPSNTKVDKKVEPKSCDKTHTGGSHHHHHH

SEQ ID NO: 87 - protein, 370 aa, Artificial Sequecne
  Synthetic construct
SDIQMTQSPSSLSASVGDRVTITCRASQGISNYLAWYQQKPGKAPKLLIYAASSLQSGVPSRFSGSRSGTDFTLTISSLQPEDFATYYCQQYGWLPLTFGQGTKVEIKGGGGSGGGGSGGGGSEISEVQLVESGGGLVQPGGSLRLSCAASGFTFSSYGMHWVRQAPGKGLEWVAVISYDGSNKYYADSVKGRFTISRDNSKNTLYLQMNSLRAEDTAVYYCARTDPYSLGGYYFDYWGQGTLVTVSSEPKSCDKTHTCPPCPGQPREPQVYTLPPSREEMTKNQVSLTCLVKGFYPSDIAVEWESNGQPENNYKTTPPVLDSDGSFFLYSKLTVDKSRWQQGNVFSCSVMHEALHNHYTQKSLSLSPGK

SEQ ID NO: 88 - protein, 480 aa, Artificial Sequence
  Synthetic construct
SDIQMTQSPSSLSASVGDRVTITCRASQGISNYLAWYQQKPGKAPKLLIYAASSLQSGVPSRFSGSRSGTDFTLTISSLQPEDFATYYCQQYGWLPLTFGQGTKVEIKGGGGSGGGGSGGGGSEISEVQLVESGGGLVQPGGSLRLSCAASGFTFSSYGMHWVRQAPGKGLEWVAVISYDGSNKYYADSVKGRFTISRDNSKNTLYLQMNSLRAEDTAVYYCARTDPYSLGGYYFDYWGQGTLVTVSSEPKSCDKTHTCPPCPAPELLGGPSVFLFPPKPKDTLMISRTPEVTCVVVDVSHEDPEVKFNWYVDGVEVHNAKTKPREEQYNSTYRVVSVLTVLHQDWLNGKEYKCKVSNKALPAPIEKTISKAKGQPREPQVYTLPPSREEMTKNQVSLTCLVKGFYPSDIAVEWESNGQPENNYKTTPPVLDSDGSFFLYSKLTVDKSRWQQGNVFSCSVMHEALHNHYTQKSLSLSPGK

SEQ ID NO: 89 - protein, 215 aa, Artificial Sequence
  Synthethic construct
SDIQMTQSPSSLSASVGDRVTITCRASQGISNYLAWYQQKPGKAPKLLIYAASSLQSGVPSRFSGSRSGTDFTLTISSLQPEDFATYYCQQYGWLPLTFGQGTKVEIKRTVAAPSVFIFPPSDEQLKSGTASVVCLLNNFYPREAKVQWKVDNALQSGNSQESVTEQDSKDSTYSLSSTLTLSKADYEKHKVYACEVTHQGLSSPVTKSFNRGEC

SEQ ID NO: 90 - protein, 455 aa, Artificial Sequence
  Synthetic contstruct
EISEVQLVESGGGLVQPGGSLRLSCAASGFTFSSYGMHWVRQAPGKGLEWVAVISYDGSNKYYADSVKGRFTISRDNSKNTLYLQMNSLRAEDTAVYYCARTDPYSLGGYYFDYWGQGTLVTVSSASTKGPSVFPLAPSSKSTSGGTAALGCLVKDYFPEPVTVSWNSGALTSGVHTFPAVLQSSGLYSLSSVVTVPSSSLGTQTYICNVNHKPSNTKVDKKVEPKSCDKTHTCPPCPAPELLGGPSVFLFPPKPKDTLMISRTPEVTCVVVDVSHEDPEVKFNWYVDGVEVHNAKTKPREEQYNSTYRVVSVLTVLHQDWLNGKEYKCKVSNKALPAPIEKTISKAKGQPREPQVYTLPPSREEMTKNQVSLTCLVKGFYPSDIAVEWESNGQPENNYKTTPPVLDSDGSFFLYSKLTVDKSRWQQGNVFSCSVMHEALHNHYTQKSLSLSPGK

SEQ ID NO: 91 - protein, 8 aa, Artificial Sequence
  Synthetic construct
QQYSYPLT

SEQ ID NO: 92 - protein, 21 aa, Artificial Sequence
  Synthetic construct
ARAPSYSYGSYHYYYYYYFDV

SEQ ID NO: 93 - protein, 9 aa, Artificial Sequence
  Synthetic construct
QQGTYLPLT

SEQ ID NO: 94 - protein, 15 aa, Artificial Sequence
  Synthetic construct
ARTYSYASRGWYFDY

SEQ ID NO: 95 - protein, 9 aa, Artificial Sequence
  Synthetic construct
QQSYRSPLT

SEQ ID NO: 96 - protein, 15 aa, Artificial Sequence
  Synthetic construct
ARSGRYGTYKGDFDY

SEQ ID NO: 97 - protein, 9 aa, Artificial Sequence
  Synthetic construct
QQSGSSPLT

SEQ ID NO: 98 - protein, 14 aa, Artificial Sequence
  Synthetic construct
ASHSYVYTAGYFDY

SEQ ID NO: 99 - protein, 9 aa, Artificial Sequence
  Synthetic construct
QQSLATPLT

SEQ ID NO: 100 - protein, 13 aa, Artificial Sequence
  Synthetic construct
ARSEYGTSGYFDY

SEQ ID NO: 101 - protein, 106 aa, Artificial Sequence
  Synthetic construct
DIVMTQSHKFMSTSVGDRVSITCKASQDVNTAVAWYQQKPGHSPKLLIYSASFRTGVPDRFTGNRSGTDFTFTISSVQAEDLAVYYCQQHYTTPPTFGGGTKLEIK

SEQ ID NO: 102 - protein, 107 aa, Artificial Sequence
  Synthetic construct
DIQMTQSPSSLSASVGDRVTITCRASQDVNTAVAWYQQKPGKAPKLLIYSASFLESGVPSRFSGSGSGTDFTLTISSLQPEDFATYYCQQHYTTPPTFGQGTKVEIK

SEQ ID NO: 103 - protein, 107 aa, Artificial Sequence [sequence omitted]

SEQ ID NO: 104 - protein, 101 aa, Artificial Sequence
  Synthetic construct
DIQMTQSPSSLSASVGDRVTITCRASQSVSSAVAWYQQKPGKAPKLLIYSASSLYSGVPSRFSGSRSGTDFTLTISSLQPEDFATYYCQQTFGQGTKVEIK

SEQ ID NO: 105 - protein, 103 aa, Artificial Sequence
  Synthetic construct
DIQMTQSPSSLSASVGDRVTITCRASQGISNYLAWYQQKPGKAPKLLIYAASSLQSGVPSRFSGSRSGTDFTLTISSLQPEDFATYYCQQPLTFGQGTKVEIK

SEQ ID NO: 106 - protein, 120 aa, Artificial Sequence
  Synthetic construct
EVQLQQSGPELVKPGASLKLSCTASGFNIKDTYIHWVKQRPEQGLEWIGRIYPTNGYTRYDPKFQDKATITADTSSNTAYLQVSRLTSEDTAVYYCSRWGGDGFYAMDYWGQGASVTVSS

SEQ ID NO: 107 - protein, 119 aa, Artificial Sequence
  Synthetic construct
EVQLVEWGGGLVQPGGSLRLSCAASGFNIKDTYIHWVRQAPGKGLEWVARIYPTNGYTRYADSVKGRFTISRDDSKNTLYQMNSLRAEDTAVYYCARWGGDGFYAMDVWGQGTLVTVSS

SEQ ID NO: 108 - protein, 119 aa, Artificial Sequence
  Synthetic construct
EVQLVEWGGGLVQPGGSLRLSCAASGFNIKDTYIHWVRQAPGKGLEWVARIYPTNGYTRYADSVKGRFTISADTSKNTAYQMNSLRAEDTAVYYCSRWGGDGFYAMDYWGQGTLVTVSS

SEQ ID NO: 109 - protein, 96 aa, Artificial Sequence
  Synthetic construct
EVQLVEWGGGLVQPGGSLRLSCAASGFNHWVRQAPGKGLEWVAITYADSVKGRFTISADTSKNTAYQMNSLRAEDTAVYYCARDYWGQGTLVTVSS

SEQ ID NO: 110 - protein, 104 aa, Artificial Sequence
  Synthetic construct
EVQLVEWGGGLVQPGGSLRLSCAASGFNHWVRQAPGKGLEWVAVISYDGSNKYYADSVKGRFTISRDNSKNTLYQMNSLRAEDTAVYYCARDYWGQGTLVTVSS

SEQ ID NO: 111 - protein, 11 aa, Artificial Sequence
  Synthetic cosntruct
RASQGISNYLA

SEQ ID NO: 112 - protein, 8 aa, Artificial Sequence
  Synthetic construct
YAASSLQS

SEQ ID NO: 113 - protein, 13 aa, Artificial Sequence
  Synthetic construct
AASQFTFSSYGMH

SEQ ID NO: 114 - protein, 10 aa, Artificial Sequence
  Synthetic construct
VISYDGSNKY

SEQ ID NO: 115 - protein, 9 aa, Artificial Sequence
  Synthetic construct
QQYGWLPLT

SEQ ID NO: 116 - protein, 15 aa, Artificial Sequence
  Synthetic construct
ARTDPYSLGGYYFDY

SEQ ID NO: 117 - protein, 6 aa, Artificial Sequence
  Synthetic construct
QGISNY

SEQ ID NO: 118 - protein, 3 aa, Artificial Sequence
  Synthetic construct
AAS

SEQ ID NO: 119 - protein, 9 aa, Artificial Sequence
  Synthetic construct
QQYGWLPLT

SEQ ID NO: 120 - protein, 8 aa, Artificial Sequence
  Synthetic construct
GFTFSSYG

SEQ ID NO: 121 - protein, 8 aa, Artificial Sequence
  Synthetic construct
ISYDGSNK

SEQ ID NO: 122 - protein, 15 aa, Artificial Sequence
  Synthetic construct
ARTDPYSLGGYYFDY